European Patent Specification EP 3 768 836 B1, published December 20, 2023. Title: ALZHEIMER'S DISEASE ANIMAL MODEL AND USE THEREOF. Applicant: Tsinghua University. The sequence listing filed with the application follows.

SEQUENCE LISTING (13 sequences)

SEQ ID NO: 1 - protein, 770 aa, Rattus norvegicus
MLPSLALLLLAAWTVRALEVPTDGNAGLLAEPQIAMFCGKLNMHMNVQNGKWESDPSGTKTCIGTKEGILQYCQEVYPELQITNVVEANQPVTIQNWCKRGRKQCKTHTHIVIPYRCLVGEFVSDALLVPDKCKFLHQERMDVCETHLHWHTVAKETCSEKSTNLHDYGMLLPCGIDKFRGVEFVCCPLAEESDSIDSADAEEDDSDVWWGGADTDYADGGEDKVVEVAEEEEVADVEEEEAEDDEDVEDGDEVEEEAEEPYEEATERTTSIATTTTTTTESVEEVVREVCSEQAETGPCRAMISRWYFDVTEGKCAPFFYGGCGGNRNNFDTEEYCMAVCGSVSSQSLLKTTSEPLPQDPVKLPTTAASTPDAVDKYLETPGDENEHAHFQKAKERLEAKHRERMSQVMREWEEAERQAKNLPKADKKAVIQHFQEKVESLEQEAANERQQLVETHMARVEAMLNDRRRLALENYITALQAVPPRPHHVFNMLKKYVRAEQKDRQHTLKHFEHVRMVDPKKAAQIRSQVMTHLRVIYERMNQSLSLLYNVPAVAEEIQDEVDELLQKEQNYSDDVLANMISEPRISYGNDALMPSLTETKTTVELLPVNGEFSLDDLQPWHPFGVDSVPANTENEVEPVDARPAADRGLTTRPGSGLTNIKTEEISEVKMDAEFGHDSGFEVRHQKLVFFAEDVGSNKGAIIGLMVGGVVIATVIVITLVMLKKKQYTSIHHGVVEVDAAVTPEERHLSKMQQNGYENPTYKFFEQMQN

SEQ ID NO: 2 - protein, 770 aa, Artificial Sequence
  mutated APP
MLPSLALLLLAAWTVRALEVPTDGNAGLLAEPQIAMFCGKLNMHMNVQNGKWESDPSGTKTCIGTKEGILQYCQEVYPELQITNVVEANQPVTIQNWCKRGRKQCKTHTHIVIPYRCLVGEFVSDALLVPDKCKFLHQERMDVCETHLHWHTVAKETCSEKSTNLHDYGMLLPCGIDKFRGVEFVCCPLAEESDSIDSADAEEDDSDVWWGGADTDYADGGEDKVVEVAEEEEVADVEEEEAEDDEDVEDGDEVEEEAEEPYEEATERTTSIATTTTTTTESVEEVVREVCSEQAETGPCRAMISRWYFDVTEGKCAPFFYGGCGGNRNNFDTEEYCMAVCGSVSSQSLLKTTSEPLPQDPVKLPTTAASTPDAVDKYLETPGDENEHAHFQKAKERLEAKHRERMSQVMREWEEAERQAKNLPKADKKAVIQHFQEKVESLEQEAANERQQLVETHMARVEAMLNDRRRLALENYITALQAVPPRPHHVFNMLKKYVRAEQKDRQHTLKHFEHVRMVDPKKAAQIRSQVMTHLRVIYERMNQSLSLLYNVPAVAEEIQDEVDELLQKEQNYSDDVLANMISEPRISYGNDALMPSLTETKTTVELLPVNGEFSLDDLQPWHPFGVDSVPANTENEVEPVDARPAADRGLTTRPGSGLTNIKTEEISEVNLDAEFRHDSGYEVHHQKLVFFAGDVGSNKGAIIGLMVGGVVIATVFVITLVMLKKKQYTSIHHGVVEVDAAVTPEERHLSKMQQNGYENPTYKFFEQMQN

SEQ ID NO: 3 - DNA, 20 bp, Artificial Sequence
  sgRNA2-target seq 1
gtacctaagagacgttgact

SEQ ID NO: 4 - DNA, 20 bp, Artificial Sequence
  sgRNA6-target seq 2
tcacggtgtcagtggagagt

SEQ ID NO: 5 - DNA, 20 bp, Artificial Sequence
  sgRNA5-target seq
gcaattagaacaacgctcca

SEQ ID NO: 6 - DNA, 20 bp, Artificial Sequence
  sgRNA1-target seq
agaacaacgctccaagggga

SEQ ID NO: 7 - DNA, 20 bp, Artificial Sequence
  sgRNA3-target seq
ccgtgtatagctagggagct

SEQ ID NO: 8 - DNA, 20 bp, Artificial Sequence
  sgRNA4-target seq
aaaacgaacattaacgacct

SEQ ID NO: 9 - DNA, 20 bp, Artificial Sequence
  sgRNA7-target seq
tccctgcttggctggtctgt

SEQ ID NO: 10 - DNA, 20 bp, Artificial Sequence
  sgRNA8-target seq
tgacatagcactgacttctg

SEQ ID NO: 11 - DNA, 20 bp, Artificial Sequence
  sgRNA9-target seq
ctgtggtaagcatccctgct

SEQ ID NO: 12 - DNA, 20 bp, Artificial Sequence
  sgRNA10-target seq
tgcccacagaccagccaagc

SEQ ID NO: 13 - protein, 9 aa, Artificial Sequence
  meganuclease motif
LAGLIDADG